European Patent Application EP 4 596 583 A1, published August 6, 2025. Title: Fusion protein and nucleic acid encoding sequence thereof, and uses of the same. Applicant: China Medical University Hospital. Application EP. The sequence listing filed with the application follows.

SEQUENCE LISTING (7 sequences)

SEQ ID NO: 1 - protein, 8 aa, synthetic construct
GVIFKNEY

SEQ ID NO: 2 - protein, 8 aa, synthetic construct
ASPGGTIT

SEQ ID NO: 3 - protein, 23 aa, synthetic construct
ALDPSTTSWSIIRHGPSLWRYSG

SEQ ID NO: 4 - protein, 370 aa, synthetic construct
MAVEGGMKCVKFLLYVLLLAFCACAVGLIAVGVGAQLVLSQTIIQGATPGSLLPVVIIAVGVFLFLVAFVGCCGACKENYCLMITFAIFLSLIMLVEVAAAIAGYVFRDKVMSEFNNNFRQQMENYPKNNHTASAHVQLVESGGGSVQAGGSLRLSCTVSGVIFKNEYMGWFRQAPGKEREGVAAASPGGTITYYGDSVKGRFTISRDNAKNTVYLQMNRLKPEDTAMYYCALDPSTTSWSIIRHGPSLWRYSGRGTQVTVSSGSSILDRMQADFKCCGAANYTDWEKIPSMSKNRVPDSCCINVTVGCGINFNEKAIHKEGCVEKIGGWLRKNVLVVAAAALGIAFVEVLGIVFACCLVKSIRSGYEVM

SEQ ID NO: 5 - DNA, 1119 bp, synthetic construct
  source 1..1119: mol_type = other DNA
atggccgtggagggcggcatgaagtgcgtgaagttcctgctgtacgtgctgctgctggccttctgcgcctgtgccgtaggccttatcgccgttggcgtgggtgcgcagctggtcctttctcagaccataatccaaggagccacccccggcagcctgctgcccgtggtgatcatcgctgtgggggtcttcctgttcctggtggccttcgtgggctgctgcggcgcctgcaaggagaactactgcctgatgatcaccttcgccatcttcctgagcctgatcatgctggtggaggtggccgccgccatcgccggctacgtgttcagagacaaggtgatgagcgagttcaacaacaacttcagacagcagatggagaactaccccaagaacaaccacaccgccagcgctcatgtgcagctggtggagtctgggggaggctcggtgcaggctggggggtctctgagactctcctgtacagtgtctggagtcatctttaagaacgagtacatgggctggttccgccaggccccagggaaggagcgcgagggggtcgcagcagcttcgcctggtggaacgattacatactatggggactccgtgaagggccgattcaccatctcccgagacaatgccaagaacacggtgtatctgcaaatgaaccgcctgaaacctgaggacactgccatgtactactgtgcgttggatccctcgactacgtcatggtctatcatccgccacggtccatcgctttggcgttatagcggccgggggacccaggtcaccgtctcctcaggatccagcatcctggacagaatgcaagccgacttcaagtgctgcggcgccgccaactacaccgactgggagaagatccctagcatgagcaagaacagagtgcccgacagctgctgcatcaacgtgaccgtgggctgcggcatcaacttcaacgagaaggccatccacaaggagggctgcgtggagaagatcggtggctggctgcgcaagaacgttctggtggtggccgccgccgccttaggcatcgccttcgtggaggtgctgggtatcgtgttcgcctgctgcctggtgaagagcatcagatccggctatgaggtaatgggcgcgccg

SEQ ID NO: 6 - protein, 128 aa, synthetic construct
HVQLVESGGGSVQAGGSLRLSCTVSGVIFKNEYMGWFRQAPGKEREGVAAASPGGTITYYGDSVKGRFTISRDNAKNTVYLQMNRLKPEDTAMYYCALDPSTTSWSIIRHGPSLWRYSGRGTQVTVSS

SEQ ID NO: 7 - DNA, 384 bp, synthetic construct
  source 1..384: mol_type = other DNA
catgtgcagctggtggagtctgggggaggctcggtgcaggctggggggtctctgagactctcctgtacagtgtctggagtcatctttaagaacgagtacatgggctggttccgccaggccccagggaaggagcgcgagggggtcgcagcagcttcgcctggtggaacgattacatactatggggactccgtgaagggccgattcaccatctcccgagacaatgccaagaacacggtgtatctgcaaatgaaccgcctgaaacctgaggacactgccatgtactactgtgcgttggatccctcgactacgtcatggtctatcatccgccacggtccatcgctttggcgttatagcggccgggggacccaggtcaccgtctcctca